European Patent Specification EP 4 095 242 B1, published August 28, 2024. Title: Novel major facilitator superfamily permease variant and a method for producing L-lysine using the same. Applicant: CJ CheilJedang Corporation. The sequence listing filed with the application follows.

SEQUENCE LISTING (10 sequences)

SEQ ID NO: 1 - protein, 481 aa, Artificial Sequence
  (H377Q)_major facilitator superfamily permease
MDSQINTQTSPAAAKLPREVVVVLSILVVSAMIMILNETILSVALPSIMEDFSVPETTAQWLTTGFMLTMAVVIPTTGYLLDRFSTKTIFVTALLFFTVGTLTAALAPTFAVLLGARIVQAVGTALVMPLLMTVTLTVVPAERRGSMMGIISIVISVAPALGPTLSGVILNSLTWHWLFWMMLPIVVIALVIGFFLIKNIGETKITPLDVLSVILSVFAFGGLVYGFSSFGAILEGEGTVGIFAIVVGAIALLIFALRQHQLGKQDKALMDLRAFKVRNFSFSLTTILLAFGAMLGTVMVLPIYLQTSLGVTALVTGLVVMPGGLLQGLISPFIGRFYDKVGPRPLLIPGAIALAIAASSMTFLNENSPVWMVVVMQVVFSIGMCLMMTPLMTTALGALPKHLYGHGSAILNTFQQLAGAAGTAIMIAALSFGTSIAASSGSAHAEAVAAGTKVAFIAGAIIAVIALVVSLFVTRVEEEAH

SEQ ID NO: 2 - DNA, 1446 bp, Artificial Sequence
  (H377Q)_NCgl2592
atggattcccaaattaatactcagacctctccggcagctgcgaagctgcctagggaggtcgttgttgttctttcgatcctcgtggtttccgcgatgatcatgattcttaatgaaaccattctgtcggttgcgttgccttccatcatggaagatttctccgtgcctgaaactactgcacagtggttgaccactggctttatgttgacgatggcagtggtgattccaactactggttatctgcttgatcgtttttccactaagacgatctttgttactgcgttgttgttctttacggttggtacgttgactgcggcgttggctccaacgtttgcggtgctgcttggtgctcgtatcgttcaggcggttggtactgcgctggtgatgcctttgctgatgacggttacgttgacggtggttcctgcggagcgtcgtggttcgatgatgggcattatttccatcgtgatttctgttgcgccggcgcttggtcctacgttgtctggtgtcattcttaactctttgacctggcactggttgttttggatgatgcttccgatcgttgttatcgctttggtaattggtttcttcttgatcaaaaatatcggcgaaaccaagatcaccccactggatgttctgtctgtcatcctttcggtgtttgccttcggtggtttggtgtacggcttcagttccttcggagcaatcctggagggcgaaggcaccgtaggtatcttcgcgatcgtcgttggcgccatcgcactcctcatctttgctttgcgacagcaccaactcggcaagcaagacaaagcactgatggatctccgagccttcaaggtgaggaacttcagcttctccttgaccaccatccttttggcgttcggcgcgatgctcggaaccgtcatggttttgccaatctacctgcagacttccctcggagttactgctttggtgaccggtttggttgttatgcccggcggcctcctccagggtctgatcagcccattcatcggacgtttctacgacaaggtcggtccacgtccgctgctgattcccggagcaattgcgctggctatcgcggcatcctcgatgactttcctcaatgagaattcacccgtgtggatggtcgtggtcatgcaagttgtgttcagcatcggcatgtgtttgatgatgacccctctcatgaccaccgctctcggcgcccttccgaagcacctctatggtcacggctccgcaattttgaacacgttccaacagctcgcaggcgcagccggaacagcgatcatgattgcagcactttccttcggcacttccattgcagcgtcttcgggatctgcgcatgctgaagctgttgccgctggtaccaaggttgcgttcatcgcaggcgcaatcatcgcggtgatcgctttggttgtttccctcttcgtcactcgcgtcgaggaagaagctcactaa

SEQ ID NO: 3 - protein, 481 aa, Artificial Sequence
  (WT)_major facilitator superfamily permease
MDSQINTQTSPAAAKLPREVVVVLSILVVSAMIMILNETILSVALPSIMEDFSVPETTAQWLTTGFMLTMAVVIPTTGYLLDRFSTKTIFVTALLFFTVGTLTAALAPTFAVLLGARIVQAVGTALVMPLLMTVTLTVVPAERRGSMMGIISIVISVAPALGPTLSGVILNSLTWHWLFWMMLPIVVIALVIGFFLIKNIGETKITPLDVLSVILSVFAFGGLVYGFSSFGAILEGEGTVGIFAIVVGAIALLIFALRQHQLGKQDKALMDLRAFKVRNFSFSLTTILLAFGAMLGTVMVLPIYLQTSLGVTALVTGLVVMPGGLLQGLISPFIGRFYDKVGPRPLLIPGAIALAIAASSMTFLNENSPVWMVVVMHVVFSIGMCLMMTPLMTTALGALPKHLYGHGSAILNTFQQLAGAAGTAIMIAALSFGTSIAASSGSAHAEAVAAGTKVAFIAGAIIAVIALVVSLFVTRVEEEAH

SEQ ID NO: 4 - DNA, 1446 bp, Artificial Sequence
  (WT)_NCgl2592
atggattcccaaattaatactcagacctctccggcagctgcgaagctgcctagggaggtcgttgttgttctttcgatcctcgtggtttccgcgatgatcatgattcttaatgaaaccattctgtcggttgcgttgccttccatcatggaagatttctccgtgcctgaaactactgcacagtggttgaccactggctttatgttgacgatggcagtggtgattccaactactggttatctgcttgatcgtttttccactaagacgatctttgttactgcgttgttgttctttacggttggtacgttgactgcggcgttggctccaacgtttgcggtgctgcttggtgctcgtatcgttcaggcggttggtactgcgctggtgatgcctttgctgatgacggttacgttgacggtggttcctgcggagcgtcgtggttcgatgatgggcattatttccatcgtgatttctgttgcgccggcgcttggtcctacgttgtctggtgtcattcttaactctttgacctggcactggttgttttggatgatgcttccgatcgttgttatcgctttggtaattggtttcttcttgatcaaaaatatcggcgaaaccaagatcaccccactggatgttctgtctgtcatcctttcggtgtttgccttcggtggtttggtgtacggcttcagttccttcggagcaatcctggagggcgaaggcaccgtaggtatcttcgcgatcgtcgttggcgccatcgcactcctcatctttgctttgcgacagcaccaactcggcaagcaagacaaagcactgatggatctccgagccttcaaggtgaggaacttcagcttctccttgaccaccatccttttggcgttcggcgcgatgctcggaaccgtcatggttttgccaatctacctgcagacttccctcggagttactgctttggtgaccggtttggttgttatgcccggcggcctcctccagggtctgatcagcccattcatcggacgtttctacgacaaggtcggtccacgtccgctgctgattcccggagcaattgcgctggctatcgcggcatcctcgatgactttcctcaatgagaattcacccgtgtggatggtcgtggtcatgcacgttgtgttcagcatcggcatgtgtttgatgatgacccctctcatgaccaccgctctcggcgcccttccgaagcacctctatggtcacggctccgcaattttgaacacgttccaacagctcgcaggcgcagccggaacagcgatcatgattgcagcactttccttcggcacttccattgcagcgtcttcgggatctgcgcatgctgaagctgttgccgctggtaccaaggttgcgttcatcgcaggcgcaatcatcgcggtgatcgctttggttgtttccctcttcgtcactcgcgtcgaggaagaagctcactaa

SEQ ID NO: 5 - DNA, 38 bp, Artificial Sequence
  NCgl2592_1F
tgaattcgagctcggtaccccggtggtttggtgtacgg

SEQ ID NO: 6 - DNA, 33 bp, Artificial Sequence
  NCgl2592_2R
cgatgctgaacacaacttgcatgaccacgacca

SEQ ID NO: 7 - DNA, 33 bp, Artificial Sequence
  NCgl2592_3F
tggtcgtggtcatgcaagttgtgttcagcatcg

SEQ ID NO: 8 - DNA, 38 bp, Artificial Sequence
  NCgl2592_4R
gtcgactctagaggatcccccgcttaaggtgaggtggc

SEQ ID NO: 9 - DNA, 18 bp, Artificial Sequence
  NCgl2592_5F
ggatgatgcttccgatcg

SEQ ID NO: 10 - DNA, 18 bp, Artificial Sequence
  NCgl2592_6R
gccgacctaccaacaagc